European Patent Specification EP 3 345 927 B1, published January 11, 2023. Title: HUMAN MONOCLONAL ANTIBODY HUMAN CD134 (OX40) AND METHODS OF MAKING AND USING SAME. Applicant: KIRIN PHARMA KABUSHIKI KAISHA KATO, SHINICHIRO SOLOFF NUGENT, RACHEL YOSHIDA, HITISHI CROFT, MICHAEL. Application TO BE ASSIGNED. The sequence listing filed with the application follows.

SEQUENCE LISTING (54 sequences)

SEQ ID NO: 1 - DNA, 1302 bp, Homo sapiens
atgtgcgtgggggctcggcggctgggccgcgggccgtgtgcggctctgctcctcctgggcctggggctgagcaccgtgacggggctccactgtgtcggggacacctaccccagcaacgaccggtgctgccacgagtgcaggccaggcaacgggatggtgagccgctgcagccgctcccagaacacggtgtgccgtccgtgcgggccgggcttctacaacgacgtggtcagctccaagccgtgcaagccctgcacgtggtgtaacctcagaagtgggagtgagcggaagcagctgtgcacggccacacaggacacagtctgccgctgccgggcgggcacccagcccctggacagctacaagcctggagttgactgtgccccctgccctccagggcacttctccccaggcgacaaccaggcctgcaagccctggaccaactgcaccttggctgggaagcacaccctgcagccggccagcaatagctcggacgcaatctgtgaggacagggaccccccagccacgcagccccaggagacccagggccccccggccaggcccatcactgtccagcccactgaagcctggcccagaacctcacagggaccctccagatcttgtgacaaaactcacacatgcccaccgtgcccagcacctgaactcctggggggaccgtcagtcttcctcttccccccaaaacccaaggacaccctcatgatctcccggacccctgaggtcacatgcgtggtggtggacgtgagccacgaagaccctgaggtcaagttcaactggtacgtggacggcgtggaggtgcataatgccaagacaaagccgcgggaggagcagtacaacagcacgtaccgtgtggtcagcgtcctcaccgtcctgcaccaggactggctgaatggcaaggagtacaagtgcaaggtctccaacaaagccctcccagcccccatcgagaaaaccatctccaaagccaaagggcagccccgagaaccacaggtgtacaccctgcccccatcccgggatgagctgaccaagaaccaggtcagcctgacctgcctggtcaaaggcttctatcccagcgacatcgccgtggagtgggagagcaatgggcagccggagaacaactacaagaccacgcctcccgtgctggactccgacggctccttcttcctctacagcaagctcaccgtggacaagagcaggtggcagcaggggaacgtcttctcatgctccgtgatgcatgaggctctgcacaaccactacacgcagaagagcctctccctgtctccgggtaaatga

SEQ ID NO: 2 - protein, 433 aa, Homo sapiens
MCVGARRLGRGPCAALLLLGLGLSTVTGLHCVGDTYPSNDRCCHECRPGNGMVSRCSRSQNTVCRPCGPGFYNDVVSSKPCKPCTWCNLRSGSERKQLCTATQDTVCRCRAGTQPLDSYKPGVDCAPCPPGHFSPGDNQACKPWTNCTLAGKHTLQPASNSSDAICEDRDPPATQPQETQGPPARPITVQPTEAWPRTSQGPSRSCDKTHTCPPCPAPELLGGPSVFLFPPKPKDTLMISRTPEVTCVVVDVSHEDPEVKFNWYVDGVEVHNAKTKPREEQYNSTYRVVSVLTVLHQDWLNGKEYKCKVSNKALPAPIEKTISKAKGQPREPQVYTLPPSRDELTKNQVSLTCLVKGFYPSDIAVEWESNGQPENNYKTTPPVLDSDGSFFLYSKLTVDKSRWQQGNVFSCSVMHEALHNHYTQKSLSLSPGK

SEQ ID NO: 3 - DNA, 420 bp, Homo sapiens
atggagtgggggccgtgctgggttttccttgttgttattttagaaggtgtccagtgtggggtgcagctggtggagtctgggggaggcttggtacagcctggggggtccctgagactctcctgtgcagcctctggattcaccttcagtagctatagcatgaactgggtccgccaggctccagggaaggggctggagtgggtttcatacattagtagtagtagtagtaccatatactatgcagactctgtgaagggccgattcaccatctccagagacaatgccaagaactcactgtatctgcaaatgaacagcctgagagacgaggacacggctgtgtattactgtgcgagaggagtgtatcacaatggctggtccttctttgactactggggccagggaaccctactcaccgtctcctca

SEQ ID NO: 4 - DNA, 390 bp, Homo sapiens
atggacatgagggtcctcgctcagctcctggggctcctgctgctctgtttcccaggtgccagatgtgacatccagatgacccagtccccatcctcactgtctgcatctgtaggaaacagagtcaccattacttgtcgggcgagtcaggatattagcagctggttagcctggtatcagcagaaaccagagaaagcccctaagtccctgatctatgctgcatccagtttgcaaagtggggtcccatcaaggttcagcggcagtggatctgggacagatttcactctcaccatcagcagcctgcagcctgaagattttgcaacttattactgccaacagtataatagttaccccctcaccttcggccaagggacacgactggagattaaacga

SEQ ID NO: 5 - DNA, 423 bp, Homo sapiens
atggacacactttgctccacgctcctgctgctgaccatcccttcatgggtcttgtcccagatcaccttgaaggagtctggtcctacgctagtgaagcccaaacagaccctcacgctgacctgcaccttctctggattctcactcagcactagtggaatgggtgtgggctggatccgtcagcccccaggaaaggccctggagtggcttgcagtcatttattgggatgatcatcaactctacagtccatctctgaagagcaggctcaccatcaccaaggacacctccaaaaaccaggtggtccttacaatgaccaacatggaccctgtggacacagccacatattactgtgcacacagacgaggggccttccagcactggggccagggcaccctggtcaccgtctcctcagcttccaccaagggc

SEQ ID NO: 6 - DNA, 387 bp, Homo sapiens
atggaaaccccagcgcagcttctcttcctcctgctactctggctcccagataccaccggagaaattgtgttgacgcagtctccaggcaccctgtctttgtctccaggggaaagagccaccctctcctgcagggccagtcagagtgttagcagcagctacttagcctggtaccagcagaaacctggccaggctcccaggctcctcatctatggtgcatccagcagggccactggcatcccagacaggttcagtggcagtgggtctgggacagacttcactctcaccatcagcagactggagcctgaagattttgcagtgtattactgtcagcagtatgatagctcgctcactttcggcggagggaccaaggtggagatcaaacgaact

SEQ ID NO: 7 - protein, 140 aa, Homo sapiens
MEWGPCWVFLVVILEGVQCGVQLVESGGGLVQPGGSLRLSCAASGFTFSSYSMNWVRQAPGKGLEWVSYISSSSSTIYYADSVKGRFTISRDNAKNSLYLQMNSLRDEDTAVYYCARGVYHNGWSFFDYWGQGTLLTVSS

SEQ ID NO: 8 - protein, 130 aa, Homo sapiens
MDMRVLAQLLGLLLLCFPGARCDIQMTQSPSSLSASVGNRVTITCRASQDISSWLAWYQQKPEKAPKSLIYAASSLQSGVPSRFSGSGSGTDFTLTISSLQPEDFATYYCQQYNSYPLTFGQGTRLEIKR

SEQ ID NO: 9 - protein, 141 aa, Homo sapiens
MDTLCSTLLLLTIPSWVLSQITLKESGPTLVKPKQTLTLTCTFSGFSLSTSGMGVGWIRQPPGKALEWLAVIYWDDHQLYSPSLKSRLTITKDTSKNQVVLTMTNMDPVDTATYYCAHRRGAFQHWGQGTLVTVSSASTKG

SEQ ID NO: 10 - protein, 129 aa, Homo sapiens
METPAQLLFLLLLWLPDTTGEIVLTQSPGTLSLSPGERATLSCRASQSVSSSYLAWYQQKPGQAPRLLIYGASSRATGIPDRFSGSGSGTDFTLTISRLEPEDFAVYYCQQYDSSLTFGGGTKVEIKRT

SEQ ID NO: 11 - DNA, 22 bp, Artificial Sequence
  Description of Artificial Sequence: Synthetic primer
ctaatacgactcactatagggc

SEQ ID NO: 12 - DNA, 31 bp, Artificial Sequence
  Description of Artificial Sequence: Synthetic primer
tcttgtccaccttggtgttgctgggcttgtg

SEQ ID NO: 13 - DNA, 30 bp, Artificial Sequence
  Description of Artificial Sequence: Synthetic primer
aggcacacaacagaggcagttccagatttc

SEQ ID NO: 14 - DNA, 18 bp, Artificial Sequence
  Description of Artificial Sequence: Synthetic primer
gtaaaacgacggccagtg

SEQ ID NO: 15 - DNA, 17 bp, Artificial Sequence
  Description of Artificial Sequence: Synthetic primer
caggaaacagctatgac

SEQ ID NO: 16 - DNA, 37 bp, Artificial Sequence
  Description of Artificial Sequence: Synthetic primer
gagagagagagctagctgaggagacggtgaccagggt

SEQ ID NO: 17 - DNA, 41 bp, Artificial Sequence
  Description of Artificial Sequence: Synthetic primer
agagagagaggtcgaccaccatggacacactttgctccacg

SEQ ID NO: 18 - DNA, 42 bp, Artificial Sequence
  Description of Artificial Sequence: Synthetic primer
agagagagagatctctcaccatggaaaccccagcgcagcttc

SEQ ID NO: 19 - DNA, 40 bp, Artificial Sequence
  Description of Artificial Sequence: Synthetic primer
agagagagagcgtacgtttgatctccaccttggtccctcc

SEQ ID NO: 20 - DNA, 25 bp, Artificial Sequence
  Description of Artificial Sequence: Synthetic primer
gctggagggcacggtcaccacgctg

SEQ ID NO: 21 - DNA, 26 bp, Artificial Sequence
  Description of Artificial Sequence: Synthetic primer
gttgaagctctttgtgacgggcgagc

SEQ ID NO: 22 - DNA, 32 bp, Artificial Sequence
  Description of Artificial Sequence: Synthetic primer
accgtgtcgactggattccaaggcatttccac

SEQ ID NO: 23 - DNA, 24 bp, Artificial Sequence
  Description of Artificial Sequence: Synthetic primer
ggtgctagctgaggagacggtgac

SEQ ID NO: 24 - DNA, 22 bp, Artificial Sequence
  Description of Artificial Sequence: Synthetic primer
aatcaagatctgtcaggacaca

SEQ ID NO: 25 - DNA, 30 bp, Artificial Sequence
  Description of Artificial Sequence: Synthetic primer
tatcccgtacgtttaatctccagtcgtgtc

SEQ ID NO: 26 - DNA, 41 bp, Artificial Sequence; identical to SEQ ID NO: 17
  Description of Artificial Sequence: Synthetic primer

SEQ ID NO: 27 - DNA, 37 bp, Artificial Sequence
  Description of Artificial Sequence: Synthetic primer
agagagagaggctagctgaagagacggtgaccattgt

SEQ ID NO: 28 - DNA, 41 bp, Artificial Sequence
  Description of Artificial Sequence: Synthetic primer
agagagagaggtcgaccaccatggaaaccccagcgcagctt

SEQ ID NO: 29 - DNA, 40 bp, Artificial Sequence
  Description of Artificial Sequence: Synthetic primer
agagagagagcgtacgtttgatttccaccttggtcccttg

SEQ ID NO: 30 - DNA, 41 bp, Artificial Sequence; identical to SEQ ID NO: 17
  Description of Artificial Sequence: Synthetic primer

SEQ ID NO: 31 - DNA, 37 bp, Artificial Sequence; identical to SEQ ID NO: 27
  Description of Artificial Sequence: Synthetic primer

SEQ ID NO: 32 - DNA, 42 bp, Artificial Sequence; identical to SEQ ID NO: 18
  Description of Artificial Sequence: Synthetic primer

SEQ ID NO: 33 - DNA, 40 bp, Artificial Sequence
  Description of Artificial Sequence: Synthetic primer
agagagagagcgtacgtttgatttccaccttggtcccctg

SEQ ID NO: 34 - DNA, 41 bp, Artificial Sequence
  Description of Artificial Sequence: Synthetic primer
agagagagaggtcgaccaccatgaccatgattacgccaagc

SEQ ID NO: 35 - DNA, 37 bp, Artificial Sequence; identical to SEQ ID NO: 16
  Description of Artificial Sequence: Synthetic primer

SEQ ID NO: 36 - DNA, 42 bp, Artificial Sequence
  Description of Artificial Sequence: Synthetic primer
agagagagagatctctcaccatggaagccccagctcagcttc

SEQ ID NO: 37 - DNA, 40 bp, Artificial Sequence
  Description of Artificial Sequence: Synthetic primer
agagagagagcgtacgtttaatctccagtcgtgtcccttg

SEQ ID NO: 38 - DNA, 408 bp, Homo sapiens
atggacacactttgctccacgctcctgctgctgaccatcccttcatgggtcttgtcccagatcaccttgaaggagtctggtcctacgctggtgaaacccacacagaccctcacgctgtcctgcaccttctctgggttctcactcagcactagtggagtgggtgtgggctggatccgtcagcccccaggaaaggccctggaatggcttgcactcattcattgggatgatgctgagcgctacagtccatctctgaagagcaggctcaccatcaccaaggacacctccaaaaaccaggtggtccttacaatgaccaacatggaccttgtggacacagccacatattactgtgcacacacccggggggcttttgatatctggggccaagggacaatggtcaccgtctcttca

SEQ ID NO: 39 - DNA, 381 bp, Homo sapiens
atggaaaccccagcgcagcttctcttcctcctgctactctggctcccagataccaccggagaaattgtgttgacgcagtctccaggcaccctgtctttgtctccaggggaaagagccatcctctcctgcagggccagtcagagtgttagcagcagcttcttagcctggtaccaacagaaacctggccaggctcccaggctcctcatctatggtgcatttagcagggccactggcatcccagacaggttcagtggcagtgggtctgggacagacttcactctcaccatcagcagactggagcctgaagattttgcagtgtattactgtcagcagtatgatagctcacggacgttcggccaggggaccaaggtggaaatcaaa

SEQ ID NO: 40 - DNA, 408 bp, Homo sapiens
atggacacactttgctccacgctcctgctgctgaccatcccttcatgggtcttgtcccagatcaccttgaaggagtctggtcctacgctggtgaaacccacacagaccctcacgctgacctgcaccttctctggattctcactcagcactagtggagtgggtgtgggctggatccgtcagcccccaggaaaggccctggagtggcttgcactcatttattgggatgatcatagcccctacagcccatctctgaagagcaggctcaccatcaccaaggacacctccaaaaaccaggtggtccttacaatgaccaacatggaccctgtggacacagccacatattactgtgcacgcacccggggggcttttgatatctggggccaagggacaatggtcaccgtctcttca

SEQ ID NO: 41 - DNA, 401 bp, Homo sapiens
atggaagccccagcgcagcttctcttcctcctgctactctggctcccagataccaccggagaaattgtgttgacacagtctccagccaccctgtctttgtctccaggggaaagagccaccctctcctgcagggccagtcagggtgttagcagctacttagcctggtaccagcagaaacctggccaggctcccaggctcctcatctatgatgcatccaacagggccactggcatcccagccaggttcagtggcagtgggcctgggacagacttcactctcaccatcagcagcctagagcctgaagattttgcagtttattactgtcagcagcgtagcaactggcatccgacgttcggccaagggaccaaggtggaaatcaaacgaactgtggctgcaccatc

SEQ ID NO: 42 - DNA, 462 bp, Homo sapiens
atgaccatgattacgccaagcttggtaccgagctcggatccactagtaacggccgccagtgtgctggaattcgcccttctaatacgactcactatagggcaagcagtggtatcaacgcagagtacggggggaggcttggtacagcctggcaggtccctgagactctcctgtgcagcctctggattcacccttgatgattatggcatgcactgggtccggcaagctccagggaagggcctggagtgggtctcaggtattagttggaatagtgatagtataggctatgtggactctgtgaagggccgattcaccatctccagagacaacgccaagaactccctgtatctgcaaatgaacagtctgagagttgaggacacggccttgtattactgtgtaaaagatattagtggctggtacagctttgactactggggccagggaaccctggtcaccgtctcctca

SEQ ID NO: 43 - DNA, 381 bp, Homo sapiens
atggaagccccagctcagcttctcttcctcctgctactctggctcccagataccaccggagaaattgtgttgacacagtctccagccaccctgtctttgtctccaggggaaagagccaccctctcctgcagggccagtcagagtgttagcagctacttagcctggtaccaacagaaacctggccaggctcccaggctcctcatctatgatgcatccaacagggccactggcatcccagccaggttcagtggcagtgggtctgggacagacttcactctcaccatcagcagcctagagcctgaagattttgcagtttattactgtcagcagcgtagcaactggccgatcaccttcggccaagggacacgactggagattaaa

SEQ ID NO: 44 - protein, 136 aa, Homo sapiens
MDTLCSTLLLLTIPSWVLSQITLKESGPTLVKPTQTLTLSCTFSGFSLSTSGVGVGWIRQPPGKALEWLALIHWDDAERYSPSLKSRLTITKDTSKNQVVLTMTNMDLVDTATYYCAHTRGAFDIWGQGTMVTVSS

SEQ ID NO: 45 - protein, 127 aa, Homo sapiens
METPAQLLFLLLLWLPDTTGEIVLTQSPGTLSLSPGERAILSCRASQSVSSSFLAWYQQKPGQAPRLLIYGAFSRATGIPDRFSGSGSGTDFTLTISRLEPEDFAVYYCQQYDSSRTFGQGTKVEIK

SEQ ID NO: 46 - protein, 136 aa, Homo sapiens
MDTLCSTLLLLTIPSWVLSQITLKESGPTLVKPTQTLTLTCTFSGFSLSTSGVGVGWIRQPPGKALEWLALIYWDDHSPYSPSLKSRLTITKDTSKNQVVLTMTNMDPVDTATYYCARTRGAFDIWGQGTMVTVSS

SEQ ID NO: 47 - protein, 127 aa, Homo sapiens
MEAPAQLLFLLLLWLPDTTGEIVLTQSPATLSLSPGERATLSCRASQGVSSYLAWYQQKPGQAPRLLIYDASNRATGIPARFSGSGPGTDFTLTISSLEPEDFAVYYCQQRSNWHPTFGQGTKVEIK

SEQ ID NO: 48 - protein, 154 aa, Homo sapiens
MTMITPSLVPSSDPLVTAASVLEFALLIRLTIGQAVVSTQSTGGGLVQPGRSLRLSCAASGFTLDDYGMHWVRQAPGKGLEWVSGISWNSDSIGYVDSVKGRFTISRDNAKNSLYLQMNSLRVEDTALYYCVKDISGWYSFDYWGQGTLVTVSS

SEQ ID NO: 49 - protein, 127 aa, Homo sapiens
MEAPAQLLFLLLLWLPDTTGEIVLTQSPATLSLSPGERATLSCRASQSVSSYLAWYQQKPGQAPRLLIYDASNRATGIPARFSGSGSGTDFTLTISSLEPEDFAVYYCQQRSNWPITFGQGTRLEIK

SEQ ID NO: 50 - protein, 277 aa, Homo sapiens
MCVGARRLGRGPCAALLLLGLGLSTVTGLHCVGDTYPSNDRCCHECRPGNGMVSRCSRSQNTVCRPCGPGFYNDVVSSKPCKPCTWCNLRSGSERKQLCTATQDTVCRCRAGTQPLDSYKPGVDCAPCPPGHFSPGDNQACKPWTNCTLAGKHTLQPASNSSDAICEDRDPPATQPQETQGPPARPITVQPTEAWPRTSQGPSTRPVEVPGGRAVAAILGLGLVLGLLGPLAILLALYLLRRDQRLPPDAHKPPGGGSFRTPIQEEQADAHSTLAKI

SEQ ID NO: 51 - protein, 203 aa, Homo sapiens
MCVGARRLGRGPCAALLLLGLGLSTVTGLHCVGDTYPSNDRCCHECRPGNGMVSRCSRSQNTVCRPCGPGFYNDVVSSKPCKPCTWCNLRSGSERKQLCTATQDTVCRCRAGTQPLDSYKPGVDCAPCPPGHFSPGDNQACKPWTNCTLAGKHTLQPASNSSDAICEDRDPPATQPQETQGPPARPITVQPTEAWPRTSQGPS

SEQ ID NO: 52 - protein, 17 aa, Homo sapiens
RPAGPGFYNDVVSSKPC

SEQ ID NO: 53 - protein, 16 aa, Homo sapiens
RAGTQPLDSYKPGVDC

SEQ ID NO: 54 - protein, 18 aa, Homo sapiens
LAGKHTLQPASNSSDAIC